European Patent Specification EP 3 224 368 B1, published October 25, 2023. Title: PROCESSES FOR CONVERSION OF BIOLOGICALLY DERIVED MEVALONIC ACID. Applicant: Visolis, Inc. Dugar, Deepak Neltner, Brian. The sequence listing filed with the application follows.

SEQUENCE LISTING (2 sequences)

SEQ ID NO: 1 - DNA, 7935 bp, Artificial Sequence
  Synthetic plasmid pSE1
gtttgacagcttatcatcgactgcacggtgcaccaatgcttctggcgtcaggcagccatcggaagctgtggtatggctgtgcaggtcgtaaatcactgcataattcgtgtcgctcaaggcgcactcccgttctggataatgttttttgcgccgacatcataacggttctggcaaatattctgaaatgagctgttgacaattaatcatccggctcgtataatgtgtggaattgtgagcggataacaatttcacacaggaaacagcgccgctgagaaaaagcgaagcggcactgctctttaacaatttatcagacaatctgtgtgggcactcgaccggaattatcgattaactttattattaaaaattaaagaggtatatattaatgtatcgattaaataaggaggaataaaccatgaaaacagtagttattattgatgcattacgaacaccaattggaaaatataaaggcagcttaagtcaagtaagtgccgtagacttaggaacacatgttacaacacaacttttaaaaagacattccactatttctgaagaaattgatcaagtaatctttggaaatgttttacaagctggaaatggccaaaatcccgcacgacaaatagcaataaacagcggtttgtctcatgaaattcccgcaatgacggttaatgaggtctgcggatcaggaatgaaggccgttattttggcgaaacaattgattcaattaggagaagcggaagttttaattgctggcgggattgagaatatgtcccaagcacctaaattacaacgttttaattacgaaacagaaagctacgatgcgcctttttctagtatgatgtatgatggattaacggatgcctttagtggtcaggcaatgggcttaactgctgaaaatgtggccgaaaagtatcatgtaactagagaagagcaagatcaattttctgtacattcacaattaaaagcagctcaagcacaagcagaagggatattcgctgacgaaatagccccattagaagtatcaggaacgcttgtggagaaagatgaagggattcgccctaattcgagcgttgagaagctaggaacgcttaaaacagtttttaaagaagacggtactgtaacagcagggaatgcatcaaccattaatgatggggcttctgctttgattattgcttcacaagaatatgccgaagcacacggtcttccttatttagctattattcgagacagtgtggaagtcggtattgatccagcctatatgggaatttcgccgattaaagccattcaaaaactgttagcgcgcaatcaacttactacggaagaaattgatctgtatgaaatcaacgaagcatttgcagcaacttcaatcgtggtccaaagagaactggctttaccagaggaaaaggtcaacatttatggtggcggtatttcattaggtcatgcgattggtgccacaggtgctcgtttattaacgagtttaagttatcaattaaatcaaaaagaaaagaaatatggagtggcttctttatgtatcggcggtggcttaggactcgctatgctactagagagacctcagcaaaaaaaaaacagccgattttatcaaatgagtcctgaggaacgcctggcttctcttcttaatgaaggccagatttctgctgatacaaaaaaagaatttgaaaatacggctttatcttcgcagattgccaatcatatgattgaaaatcaaatcagtgaaacagaagtgccgatgggcgttggcttacatttaacagtggacgaaactgattatttggtaccaatggcgacagaagagccctcagttattgcggctttgagtaatggtgcaaaaatagcacaaggatttaaaacagtgaatcaacaacgcttaatgcgtggacaaatcgttttttacgatgttgcagatcccgagtcattgattgataaactacaagtaagagaagcggaagtttttcaacaagcagagttaagttatccatctatcgttaaacggggcggcggcttaagagatttgcaatatcgtacttttgatgaatcatttgtatctgtcgactttttagtagatgttaaggatgcaatgggggcaaatatcgttaacgctatgttggaaggtgtggccgagttgttccgtgaatggtttgcggagcaaaagattttattcagtattttaagtaattatgccacggagtcggttgttacgatgaaaacggctattccagtttcacgtttaagtaaggggagcaatggccgggaaattgctgaaaaaattgttttagcttcacgctatgcttcattagatccttatcgggcagtcacgcataacaaaggaatcatgaatggcattgaagctgtagttttagctacaggaaatgatacacgcgctgttagcgcttcttgtcatgcttttgcggtgaaggaaggtcgctaccaaggcttgactagttggacgctggatggcgaacaactaattggtgaaatttcagttccgcttgctttagccacggttggcggtgccacaaaagtcttacctaaatctcaagcagctgctgatttgttagcagtgacggatgcaaaagaactaagtcgagtagtagcggctgttggtttggcacaaaatttagcggcgttacgggccttagtctctgaaggaattcaaaaaggacacatggctctacaagcacgttctttagcgatgacggtcggagctactggtaaagaagttgaggcagtcgctcaacaattaaaacgtcaaaaaacgatgaaccaagaccgagccatggctattttaaatgatttaagaaaacaataagatctaaggagttaaagaaatgacaattgggattgataaaattagtttttttgtgcccccttattatattgatatgacggcactggctgaagccagaaatgtagaccctggaaaatttcatattggtattgggcaagaccaaatggcggtgaacccaatcagccaagatattgtgacatttgcagccaatgccgcagaagcgatcttgaccaaagaagataaagaggccattgatatggtgattgtcgggactgagtccagtatcgatgagtcaaaagcggccgcagttgtcttacatcgtttaatggggattcaacctttcgctcgctctttcgaaatcaaggaaggttgttacggagcaacagcaggcttacagttagctaagaatcacgtagccttacatccagataaaaaagtcttggtcgtagcggcagatattgcaaaatatggcttaaattctggcggtgagcctacacaaggagctggggcggttgcaatgttagttgctagtgaaccgcgcattttggctttaaaagaggataatgtgatgctgacgcaagatatctatgacttttggcgtccaacaggccacccgtatcctatggtcgatggtcctttgtcaaacgaaacctacatccaatcttttgcccaagtctgggatgaacataaaaaacgaaccggtcttgattttgcagattatgatgctttagcgttccatattccttacacaaaaatgggcaaaaaagccttattagcaaaaatctccgaccaaactgaagcagaacaggaacgaattttagcccgttatgaagaaagtatcgtctatagtcgtcgcgtaggaaacttgtatacgggttcactttatctgggactcatttcccttttagaaaatgcaacgactttaaccgcaggcaatcaaattggtttattcagttatggttctggtgctgtcgctgaatttttcactggtgaattagtagctggttatcaaaatcatttacaaaaagaaactcatttagcactgctggataatcggacagaactttctatcgctgaatatgaagccatgtttgcagaaactttagacacagacattgatcaaacgttagaagatgaattaaaatatagtatttctgctattaataataccgttcgttcttatcgaaactaatctagaacaaaaactcatctcagaagaggatctgaatagcgccgtcgaccatcatcatcatcatcattgagtttaaacggtctccagcttggctgttttggcggatgagagaagattttcagcctgatacagattaaatcagaacgcagaagcggtctgataaaacagaatttgcctggcggcagtagcgcggtggtcccacctgaccccatgccgaactcagaagtgaaacgccgtagcgccgatggtagtgtggggtctccccatgcgagagtagggaactgccaggcatcaaataaaacgaaaggctcagtcgaaagactgggcctttcgttttatctgttgtttgtcggtgaacgctctcctgagtaggacaaatccgccgggagcggatttgaacgttgcgaagcaacggcccggagggtggcgggcaggacgcccgccataaactgccaggcatcaaattaagcagaaggccatcctgacggatggcctttttgcgtttctacaaactctttttgtttatttttctaaatacattcaaatatgtatccgctcatgagacaataaccctgataaatgcttcaataatattgaaaaaggaagagtatgagtattcaacatttccgtgtcgcccttattcccttttttgcggcattttgccttcctgtttttgctcacccagaaacgctggtgaaagtaaaagatgctgaagatcagttgggtgcacgagtgggttacatcgaactggatctcaacagcggtaagatccttgagagttttcgccccgaagaacgttttccaatgatgagcacttttaaagttctgctatgtggcgcggtattatcccgtgttgacgccgggcaagagcaactcggtcgccgcatacactattctcagaatgacttggttgagtactcaccagtcacagaaaagcatcttacggatggcatgacagtaagagaattatgcagtgctgccataaccatgagtgataacactgcggccaacttacttctgacaacgatcggaggaccgaaggagctaaccgcttttttgcacaacatgggggatcatgtaactcgccttgatcgttgggaaccggagctgaatgaagccataccaaacgacgagcgtgacaccacgatgcctgtagcaatggcaacaacgttgcgcaaactattaactggcgaactacttactctagcttcccggcaacaattaatagactggatggaggcggataaagttgcaggaccacttctgcgctcggcccttccggctggctggtttattgctgataaatctggagccggtgagcgtgggtctcgcggtatcattgcagcactggggccagatggtaagccctcccgtatcgtagttatctacacgacggggagtcaggcaactatggatgaacgaaatagacagatcgctgagataggtgcctcactgattaagcattggtaactgtcagaccaagtttactcatatatactttagattgatttaaaacttcatttttaatttaaaaggatctaggtgaagatcctttttgataatctcatgaccaaaatcccttaacgtgagttttcgttccactgagcgtcagaccccgtagaaaagatcaaaggatcttcttgagatcctttttttctgcgcgtaatctgctgcttgcaaacaaaaaaaccaccgctaccagcggtggtttgtttgccggatcaagagctaccaactctttttccgaaggtaactggcttcagcagagcgcagataccaaatactgtccttctagtgtagccgtagttaggccaccacttcaagaactctgtagcaccgcctacatacctcgctctgctaatcctgttaccagtggctgctgccagtggcgataagtcgtgtcttaccgggttggactcaagacgatagttaccggataaggcgcagcggtcgggctgaacggggggttcgtgcacacagcccagcttggagcgaacgacctacaccgaactgagatacctacagcgtgagctatgagaaagcgccacgcttcccgaagggagaaaggcggacaggtatccggtaagcggcagggtcggaacaggagagcgcacgagggagcttccagggggaaacgcctggtatctttatagtcctgtcgggtttcgccacctctgacttgagcgtcgatttttgtgatgctcgtcaggggggcggagcctatggaaaaacgccagcaacgcggcctttttacggttcctggccttttgctggccttttgctcacatgttctttcctgcgttatcccctgattctgtggataaccgtattaccgcctttgagtgagctgataccgctcgccgcagccgaacgaccgagcgcagcgagtcagtgagcgaggaagcggaagagcgcctgatgcggtattttctccttacgcatctgtgcggtatttcacaccgcatatggtgcactctcagtacaatctgctctgatgccgcatagttaagccagtatacactccgctatcgctacgtgactgggtcatggctgcgccccgacacccgccaacacccgctgacgcgccctgacgggcttgtctgctcccggcatccgcttacagacaagctgtgaccgtctccgggagctgcatgtgtcagaggttttcaccgtcatcaccgaaacgcgcgaggcagcagatcaattcgcgcgcgaaggcgaagcggcatgcatttacgttgacaccatcgaatggtgcaaaacctttcgcggtatggcatgatagcgcccggaagagagtcaattcagggtggtgaatgtgaaaccagtaacgttatacgatgtcgcagagtatgccggtgtctcttatcagaccgtttcccgcgtggtgaaccaggccagccacgtttctgcgaaaacgcgggaaaaagtggaagcggcgatggcggagctgaattacattcccaaccgcgtggcacaacaactggcgggcaaacagtcgttgctgattggcgttgccacctccagtctggccctgcacgcgccgtcgcaaattgtcgcggcgattaaatctcgcgccgatcaactgggtgccagcgtggtggtgtcgatggtagaacgaagcggcgtcgaagcctgtaaagcggcggtgcacaatcttctcgcgcaacgcgtcagtgggctgatcattaactatccgctggatgaccaggatgccattgctgtggaagctgcctgcactaatgttccggcgttatttcttgatgtctctgaccagacacccatcaacagtattattttctcccatgaagacggtacgcgactgggcgtggagcatctggtcgcattgggtcaccagcaaatcgcgctgttagcgggcccattaagttctgtctcggcgcgtctgcgtctggctggctggcataaatatctcactcgcaatcaaattcagccgatagcggaacgggaaggcgactggagtgccatgtccggttttcaacaaaccatgcaaatgctgaatgagggcatcgttcccactgcgatgctggttgccaacgatcagatggcgctgggcgcaatgcgcgccattaccgagtccgggctgcgcgttggtgcggatatctcggtagtgggatacgacgataccgaagacagctcatgttatatcccgccgtcaaccaccatcaaacaggattttcgcctgctggggcaaaccagcgtggaccgcttgctgcaactctctcagggccaggcggtgaagggcaatcagctgttgcccgtctcactggtgaaaagaaaaaccaccctggcgcccaatacgcaaaccgcctctccccgcgcgttggccgattcattaatgcagctggcacgacaggtttcccgactggaaagcgggcagtgagcgcaacgcaattaatgtgagttagcgcgaattgatctg

SEQ ID NO: 2 - DNA, 10857 bp, Artificial Sequence
  Synthetic plasmid pVS19
gacgaaagggcctcgtgatacgcctatttttataggttaatgtcatgataataatggtttcttagatgatccaatatcaaaggaaatgatagcattgaaggatgagactaatccaattgaggagtggcagcatatagaacagctaaagggtagtgctgaaggaagcatacgataccccgcatggaatgggataatatcacaggaggtactagactacctttcatcctacataaatagacgcatataagtacgcatttaagcataaacacgcactatgccgttcttctcatgtatatatatatacaggcaacacgcagatataggtgcgacgtgaacagtgagctgtatgtgcgcagctcgcgttgcattttcggaagcgctcgttttcggaaacgctttgaagttcctattccgaagttcctattctctagctagaaagtataggaacttcagagcgcttttgaaaaccaaaagcgctctgaagacgcactttcaaaaaaccaaaaacgcaccggactgtaacgagctactaaaatattgcgaataccgcttccacaaacattgctcaaaagtatctctttgctatatatctctgtgctatatccctatataacctacccatccacctttcgctccttgaacttgcatctaaactcgacctctacattttttatgtttatctctagtattactctttagacaaaaaaattgtagtaagaactattcatagagtgaatcgaaaacaatacgaaaatgtaaacatttcctatacgtagtatatagagacaaaatagaagaaaccgttcataattttctgaccaatgaagaatcatcaacgctatcactttctgttcacaaagtatgcgcaatccacatcggtatagaatataatcggggatgcctttatcttgaaaaaatgcacccgcagcttcgctagtaatcagtaaacgcgggaagtggagtcaggctttttttatggaagagaaaatagacaccaaagtagccttcttctaaccttaacggacctacagtgcaaaaagttatcaagagactgcattatagagcgcacaaaggagaaaaaaagtaatctaagatgctttgttagaaaaatagcgctctcgggatgcatttttgtagaacaaaaaagaagtatagattctttgttggtaaaatagcgctctcgcgttgcatttctgttctgtaaaaatgcagctcagattctttgtttgaaaaattagcgctctcgcgttgcatttttgttttacaaaaatgaagcacagattcttcgttggtaaaatagcgctttcgcgttgcatttctgttctgtaaaaatgcagctcagattctttgtttgaaaaattagcgctctcgcgttgcatttttgttctacaaaatgaagcacagatgcttcgttcaggtggcacttttcggggaaatgtgcgcggaacccctatttgtttatttttctaaatacattcaaatatgtatccgctcatgagacaataaccctgataaatgcttcaataatattgaaaaaggaagagtatgagtattcaacatttccgtgtcgcccttattcccttttttgcggcattttgccttcctgtttttgctcacccagaaacgctggtgaaagtaaaagatgctgaagatcagttgggtgcacgagtgggttacatcgaactggatctcaacagcggtaagatccttgagagttttcgccccgaagaacgttttccaatgatgagcacttttaaagttctgctatgtggcgcggtattatcccgtattgacgccgggcaagagcaactcggtcgccgcatacactattctcagaatgacttggttgagtactcaccagtcacagaaaagcatcttacggatggcatgacagtaagagaattatgcagtgctgccataaccatgagtgataacactgcggccaacttacttctgacaacgatcggaggaccgaaggagctaaccgcttttttgcacaacatgggggatcatgtaactcgccttgatcgttgggaaccggagctgaatgaagccataccaaacgacgagcgtgacaccacgatgcctgtagcaatggcaacaacgttgcgcaaactattaactggcgaactacttactctagcttcccggcaacaattaatagactggatggaggcggataaagttgcaggaccacttctgcgctcggcccttccggctggctggtttattgctgataaatctggagccggtgagcgtgggtctcgcggtatcattgcagcactggggccagatggtaagccctcccgtatcgtagttatctacacgacggggagtcaggcaactatggatgaacgaaatagacagatcgctgagataggtgcctcactgattaagcattggtaactgtcagaccaagtttactcatatatactttagattgatttaaaacttcatttttaatttaaaaggatctaggtgaagatcctttttgataatctcatgaccaaaatcccttaacgtgagttttcgttccactgagcgtcagaccccgtagaaaagatcaaaggatcttcttgagatcctttttttctgcgcgtaatctgctgcttgcaaacaaaaaaaccaccgctaccagcggtggtttgtttgccggatcaagagctaccaactctttttccgaaggtaactggcttcagcagagcgcagataccaaatactgttcttctagtgtagccgtagttaggccaccacttcaagaactctgtagcaccgcctacatacctcgctctgctaatcctgttaccagtggctgctgccagtggcgataagtcgtgtcttaccgggttggactcaagacgatagttaccggataaggcgcagcggtcgggctgaacggggggttcgtgcacacagcccagcttggagcgaacgacctacaccgaactgagatacctacagcgtgagctatgagaaagcgccacgcttcccgaagggagaaaggcggacaggtatccggtaagcggcagggtcggaacaggagagcgcacgagggagcttccagggggaaacgcctggtatctttatagtcctgtcgggtttcgccacctctgacttgagcgtcgatttttgtgatgctcgtcaggggggcggagcctatggaaaaacgccagcaacgcggcctttttacggttcctggccttttgctggccttttgctcacatgttctttcctgcgttatcccctgattctgtggataaccgtattaccgcctttgagtgagctgataccgctcgccgcagccgaacgaccgagcgcagcgagtcagtgagcgaggaagcggaagagcgcccaatacgcaaaccgcctctccccgcgcgttggccgattcattaatgcagctggcacgacaggtttcccgactggaaagcgggcagtgagcgcaacgcaattaatgtgagttagctcactcattaggcaccccaggctttacactttatgcttccggctcgtatgttgtgtggaattgtgagcggataacaatttcacacaggaaacagctatgaccatgattacgccaagcgcgcaattaaccctcactaaagggaacaaaagctggagctcaccggtatacccgggaaacagctgagtttatcattatcaatactcgccatttcaaagaatacgtaaataattaatagtagtgattttcctaactttatttagtcaaaaaattagccttttaattctgctgtaacccgtacatgcccaaaatagggggcgggttacacagaatatataacatcgtaggtgtctgggtgaacagtttattcctggcatccactaaatataatggagcccgctttttaagctggcatccagaaaaaaaaagaatcccagcaccaaaatattgttttcttcaccaaccatcagttcataggtccattctcttagcgcaactacagagaacaggggcacaaacaggcaaaaaacgggcacaacctcaatggagtgatgcaacctgcctggagtaaatgatgacacaaggcaattgacccacgcatgtatctatctcattttcttacaccttctattaccttctgctctctctgatttggaaaaagctgaaaaaaaaggttgaaaccagttccctgaaattattcccctacttgactaataagtatataaagacggtaggtattgattgtaattctgtaaatctatttcttaaacttcttaaattctacttttatagttagtcttttttttagttttaaaacaccagaacttagtttcgacggattggcggccgctaaaatcatggctagcaagacggtcgtcattattgacgcacttcgtactcctattggtaaatacaaaggttctttgtctcaagtttccgctgttgatttgggtactcatgtcaccacacagttgcttaaacgtcactctacaatttctgaggaaattgaccaggttatttttggtaacgttttgcaagccggcaatggtcaaaacccagctcgtcaaattgccattaatagtggactttctcatgaaattccagctatgactgtgaacgaagtttgcggatctggcatgaaagcagttattttggcaaaacaacttatccaacttggagaagctgaggtgttgatcgcaggtggcatcgaaaatatgtctcaggctccaaaattgcaacgttttaactacgaaacggagtcttacgatgccccatttagttctatgatgtacgacggtttgacagatgcattttccggtcaagcaatgggtttgaccgccgaaaatgtcgctgaaaagtatcatgtgacgcgtgaagaacaagaccaattttccgtccatagtcaacttaaagctgcccaagctcaggcagaaggtatttttgccgatgaaatcgcccctcttgaggtttccggtacacttgttgagaaagatgaaggtattcgtcctaatagttccgtcgaaaagttgggaacacttaagactgtcttcaaggaggatggaacggtgacagcaggtaacgcttctacaattaatgatggtgcatctgctttgattattgcctcccaagaatatgctgaagcacatggtttgccatatttggccatcatccgtgactccgttgaggtcggcattgatcctgcctatatgggcatttccccaatcaaggcaattcaaaagttgttggctcgtaatcaacttacaactgaagagattgatctttatgagatcaatgaggcctttgctgccacttccattgttgttcagcgtgaattggctttgcctgaagaaaaagtgaacatttacggaggtggaatctctttgggacatgcaatcggcgcaaccggcgcacgtcttttgacctctctttcttatcagttgaatcaaaaggaaaaaaagtacggtgtggctagtttgtgtattggaggtggcttgggattggcaatgttgttggagcgtcctcaacaaaagaaaaactcccgtttctatcagatgagtcctgaagaacgtcttgcttccttgttgaatgagggccagattagtgctgatacgaagaaagagttcgaaaacaccgcactttcttctcagattgctaaccacatgattgaaaatcagatttccgaaactgaagttccaatgggagtgggattgcatttgactgttgacgagactgattatttggtgccaatggctactgaagaaccatctgtgatcgccgccctttctaacggtgcaaagattgctcagggatttaaaactgtcaatcagcaacgtcttatgcgtggacagatcgttttctacgatgtcgcagaccctgagtcccttattgataaacttcaagttcgtgaagctgaagtcttccagcaagcagaacttagttatccttctatcgtcaaacgtggtggcggcttgcgtgatttgcaatatcgtactttcgacgagagttttgttagtgtggattttttggttgatgtgaaggacgcaatgggtgcaaatatcgttaacgcaatgttggaaggcgttgctgaattgtttcgtgaatggttcgccgaacaaaagattttgttctccattttgtccaattacgctacagaatctgttgtcacaatgaagactgccatccctgtgtctcgtttgtctaaaggtagtaacggtcgtgaaattgcagaaaaaatcgtgttggcaagtcgttatgctagtcttgatccatatcgtgccgttacgcacaataaaggtatcatgaacggtatcgaagctgtggtcttggccaccggcaatgatacacgtgctgtcagtgcaagttgtcatgcatttgcagttaaagaaggtcgttaccaaggattgacttcctggactttggatggtgagcaacttattggcgaaatttctgttccattggctcttgctaccgttggtggtgccacaaaagttcttccaaagtctcaagctgccgctgacttgttggctgttaccgacgctaaagagcttagtcgtgttgttgcagctgtcggtttggctcaaaatttggctgcattgcgtgccttggttagtgaaggtatccaaaaaggtcacatggccttgcaagctcgttccttggctatgaccgttggagctacaggtaaggaagtggaagctgttgcacaacagttgaagcgtcaaaaaactatgaatcaagatcgtgctatggccattttgaatgatttgcgtaaacaactcgagtaatgatcagcgaatttcttatgatttatgatttttattattaaataagttataaaaaaaataagtgtatacaaattttaaagtgactcttaggttttaaaacgaaaattcttattcttgagtaactctttcctgtaggtcaggttgctttctcaggtatagcatgaggtcgctcttatcgccgggaaacagctgatagcttcaaaatgtttctactccttttttactcttccagattttctcggactccgcgcatcgccgtaccacttcaaaacacccaagcacagcatactaaatttcccctctttcttcctctagggtgtcgttaattacccgtactaaaggtttggaaaagaaaaaagagaccgcctcgtttctttttcttcgtcgaaaaaggcaataaaaatttttatcacgtttctttttcttgaaaattttttttttgatttttttctctttcgatgacctcccattgatatttaagttaataaacggtcttcaatttctcaagtttcagtttcatttttcttgttctattacaactttttttacttcttgctcattagaaagaaagcatagcaatctaatctaagttttggcggccgctaaaatcatggctagcaccatcggcatcgacaagatttctttcttcgttccaccatattacattgacatgacggctttggctgaagcccgtaacgttgatcctggtaaattccatattggaatcggccaggaccaaatggctgtgaatccaatcagtcaagatattgtcactttcgcagcaaacgccgcagaagccattttgactaaagaggataaggaagctattgacatggttattgtcggcactgaaagttccattgatgaatctaaggcagctgctgtcgttcttcatcgtcttatgggtattcaaccatttgcacgtagttttgaaattaaagagggatgttatggagcaaccgcaggcttgcagttggcaaaaaatcatgtggctttgcatccagataaaaaggttttggttgttgcagccgatattgctaagtacggattgaatagtggtggtgagccaacgcaaggtgcaggagctgttgcaatgttggttgctagtgaacctcgtatccttgccttgaaggaagataacgtcatgttgacccaggatatttatgatttttggcgtccaacaggccatccttaccctatggtcgatggtcctcttagtaatgaaacatacattcaatcttttgcccaagtctgggatgaacacaaaaagcgtacaggtcttgattttgccgattatgatgcccttgctttccacattccttacactaaaatgggtaagaaagcattgttggctaaaatttctgaccaaactgaagccgaacaggaacgtatcttggctcgttatgaagaatctatcgtgtactctcgtcgtgtgggtaacctttatacaggttctctttatcttggattgatttccttgcttgagaatgctactactttgacggctggaaatcagatcggtttgttttcctatggttctggcgctgttgctgagttttttacaggtgaattggttgcaggttaccaaaatcacttgcaaaaagagacacatcttgctttgttggataatcgtaccgaattgtctatcgctgaatatgaagcaatgttcgctgagactttggacacagatattgaccaaacccttgaggacgaattgaaatattccatctccgccattaacaatactgtgcgttcctaccgtaacctcgagtaatgatcatctctgcttttgtgcgcgtatgtttatgtatgtacctctctctctatttctatttttaaaccaccctctcaataaaataaaaataataaagtatttttaaggaaaagacgtgtttaagcactgactttatctactttttgtacgttttcattgatataatgtgttttgtctctcccttttctacgaaaatttcaaaaattgaccaaaaaaaggaatatatatacgaaaaactattatatttatatatcatagtgttgataaaaaatgtttatccattggaccgtgtatcatatttatcgccggcgaataaattaaggcgcgccaacatatccggaggtacccaattcgccctatagtgagtcgtattacgcgcgctcactggccgtcgttttacaacgtcgtgactgggaaaaccctggcgttacccaacttaatcgccttgcagcacatccccctttcgccagctggcgtaatagcgaagaggcccgcaccgatcgcccttcccaacagttgcgcagcctgaatggcgaatggacgcgccctgtagcggcgcattaagcgcggcgggtgtggtggttacgcgcagcgtgaccgctacacttgccagcgccctagcgcccgctcctttcgctttcttcccttcctttctcgccacgttcgccggctttccccgtcaagctctaaatcgggggctccctttagggttccgatttagtgctttacggcacctcgaccccaaaaaacttgattagggtgatggttcacgtagtgggccatcgccctgatagacggtttttcgccctttgacgttggagtccacgttctttaatagtggactcttgttccaaactggaacaacactcaaccctatctcggtctattcttttgatttataagggattttgccgatttcggcctattggttaaaaaatgagctgatttaacaaaaatttaacgcgaattttaacaaaatattaacgcttacaatttcctgatgcggtattttctccttacgcatctgtgcggtatttcacaccgcatagggtaataactgatataattaaattgaagctctaatttgtgagtttagtatacatgcatttacttataatacagttttttagttttgctggccgcatcttctcaaatatgcttcccagcctgcttttctgtaacgttcaccctctaccttagcatcccttccctttgcaaatagtcctcttccaacaataataatgtcagatcctgtagagaccacatcatccacggttctatactgttgacccaatgcgtctcccttgtcatctaaacccacaccgggtgtcataatcaaccaatcgtaaccttcatctcttccacccatgtctctttgagcaataaagccgataacaaaatctttgtcgctcttcgcaatgtcaacagtacccttagtatattctccagtagatagggagcccttgcatgacaattctgctaacatcaaaaggcctctaggttcctttgttacttcttctgccgcctgcttcaaaccgctaacaatacctggtcccaccacaccgtgtgcattcgtaatgtctgcccattctgctattctgtatacacccgcagagtactgcaatttgactgtattaccaatgtcagcaaattttctgtcttcgaagagtaaaaaattgtacttggcggataatgcctttagcggcttaactgtgccctccatggaaaaatcagtcaagatatccacatgtgtttttagtaaacaaattttgggacctaatgcttcaactaactccagtaattccttggtggtacgaacatccaatgaagcacacaagtttgtttgcttttcgtgcatgatattaaatagcttggcagcaacaggactaggatgagtagcagcacgttccttatatgtagctttcgacatgatttatcttcgtttcctgcatgtttttgttctgtgcagttgggttaagaatactgggcaatttcatgtttcttcaacactacatatgcgtatatataccaatctaagtctgtgctccttccttcgttcttccttctgttcggagattaccgaatcaaaaaaatttcaaggaaaccgaaatcaaaaaaaagaataaaaaaaaaatgatgaattgaaaaggtggtatggtgcactctcagtacaatctgctctgatgccgcatagttaagccagccccgacacccgccaacacccgctgacgcgccctgacgggcttgtctgctcccggcatccgcttacagacaagctgtgaccgtctccgggagctgcatgtgtcagaggttttcaccgtcatcaccgaaacgcgcga